European Patent Application EP 4 431 943 A2, published September 18, 2024. Title: METHODS FOR IDENTIFYING ANTIGEN-SPECIFIC T CELL RECEPTORS. Applicant: MEMORIAL SLOAN-KETTERING CANCER CENTER. Application EM. The sequence listing filed with the application follows.

SEQUENCE LISTING (66 sequences)

SEQ ID NO: 1 - protein, 27 aa, synthetic construct
  REGION 1..27: note = Description of Artificial Sequence: Synthetic peptide
RAKRSGSGATNFSLLKQAGDVEENPGP

SEQ ID NO: 2 - DNA, 81 bp, synthetic construct
  misc_feature 1..81: note = Description of Artificial Sequence: Synthetic oligonucleotide
  source 1..81: mol_type = other DNA
agggcaaagaggagcggatccggagccaccaatttctctctgctgaagcaggcaggcgatgtggaggagaacccaggacct

SEQ ID NO: 3 - DNA, 81 bp, synthetic construct
  misc_feature 1..81: note = Description of Artificial Sequence: Synthetic oligonucleotide
  source 1..81: mol_type = other DNA
agggcaaagcggagcggaagtggcgccaccaatttctccctgctgaaacaggccggggatgtcgaggaaaatcccggacct

SEQ ID NO: 4 - protein, 4 aa, synthetic construct
  REGION 1..4: note = Description of Artificial Sequence: Synthetic peptide
SGSG

SEQ ID NO: 5 - protein, 65 aa, synthetic construct
  REGION 1..65: note = Description of Artificial Sequence: Synthetic polypeptide
HAGLSNRLARDNELRENDKEQLKAISTRDPLSEITEQEKDFLWSHRHYCVTIPEILPKLLLSVKW

SEQ ID NO: 6 - protein, 65 aa, synthetic construct
  REGION 1..65: note = Description of Artificial Sequence: Synthetic polypeptide
HAGLSNRLARDNELRENDKEQLKAISTRDPLSKITEQEKDFLWSHRHYCVTIPEILPKLLLSVKW

SEQ ID NO: 7 - protein, 65 aa, synthetic construct
  REGION 1..65: note = Description of Artificial Sequence: Synthetic polypeptide
LSNRLARDNELRENDKEQLKAISTRDPLSEITEQEKDFLWSHRHYCVTIPEILPKLLLSVKWNSR

SEQ ID NO: 8 - protein, 65 aa, synthetic construct
  REGION 1..65: note = Description of Artificial Sequence: Synthetic polypeptide
LSNRLARDNELRENDKEQLKAISTRDPLSEITKQEKDFLWSHRHYCVTIPEILPKLLLSVKWNSR

SEQ ID NO: 9 - protein, 45 aa, synthetic construct
  REGION 1..45: note = Description of Artificial Sequence: Synthetic polypeptide
KTLALDKTEQEALEYFMKQMNDAHHGGWTTKMDWIFHTIKQHALN

SEQ ID NO: 10 - protein, 45 aa, synthetic construct
  REGION 1..45: note = Description of Artificial Sequence: Synthetic polypeptide
KTLALDKTEQEALEYFMKQMNDARHGGWTTKMDWIFHTIKQHALN

SEQ ID NO: 11 - protein, 45 aa, synthetic construct
  REGION 1..45: note = Description of Artificial Sequence: Synthetic polypeptide
KTLALDKTEQEALEYFMKQMNDALHGGWTTKMDWIFHTIKQHALN

SEQ ID NO: 12 - protein, 25 aa, synthetic construct
  REGION 1..25: note = Description of Artificial Sequence: Synthetic peptide
GHSYTTAEELAGIGILTVILGVLLL

SEQ ID NO: 13 - protein, 15 aa, synthetic construct
  REGION 1..15: note = Description of Artificial Sequence: Synthetic peptide
CAVRPLYGGSYIPTF

SEQ ID NO: 14 - protein, 12 aa, synthetic construct
  REGION 1..12: note = Description of Artificial Sequence: Synthetic peptide
CAVNFGGGKLIF

SEQ ID NO: 15 - protein, 13 aa, synthetic construct
  REGION 1..13: note = Description of Artificial Sequence: Synthetic peptide
CVLGGGSARQLTF

SEQ ID NO: 16 - protein, 13 aa, synthetic construct
  REGION 1..13: note = Description of Artificial Sequence: Synthetic peptide
CAVNKRSNYQLIW

SEQ ID NO: 17 - protein, 12 aa, synthetic construct
  REGION 1..12: note = Description of Artificial Sequence: Synthetic peptide
CVVNDGTYKYIF

SEQ ID NO: 18 - protein, 11 aa, synthetic construct
  REGION 1..11: note = Description of Artificial Sequence: Synthetic peptide
CAASMIARLMF

SEQ ID NO: 19 - protein, 15 aa, synthetic construct
  REGION 1..15: note = Description of Artificial Sequence: Synthetic peptide
CAMRDFSGGYNKLIF

SEQ ID NO: 20 - protein, 11 aa, synthetic construct
  REGION 1..11: note = Description of Artificial Sequence: Synthetic peptide
CAGHPLNDMRF

SEQ ID NO: 21 - protein, 13 aa, synthetic construct
  REGION 1..13: note = Description of Artificial Sequence: Synthetic peptide
CAFVRNNNARLMF

SEQ ID NO: 22 - protein, 15 aa, synthetic construct
  REGION 1..15: note = Description of Artificial Sequence: Synthetic peptide
CAESLMDTGRRALTF

SEQ ID NO: 23 - protein, 14 aa, synthetic construct
  REGION 1..14: note = Description of Artificial Sequence: Synthetic peptide
CASSYVGNTGELFF

SEQ ID NO: 24 - protein, 13 aa, synthetic construct
  REGION 1..13: note = Description of Artificial Sequence: Synthetic peptide
CASSLSFGTEAFF

SEQ ID NO: 25 - protein, 12 aa, synthetic construct
  REGION 1..12: note = Description of Artificial Sequence: Synthetic peptide
CASSRMNTEAFF

SEQ ID NO: 26 - protein, 14 aa, synthetic construct
  REGION 1..14: note = Description of Artificial Sequence: Synthetic peptide
CASSYFQGAAEAFF

SEQ ID NO: 27 - protein, 13 aa, synthetic construct
  REGION 1..13: note = Description of Artificial Sequence: Synthetic peptide
CASSPKQQYEQYF

SEQ ID NO: 28 - protein, 15 aa, synthetic construct
  REGION 1..15: note = Description of Artificial Sequence: Synthetic peptide
CASSFTTGVGTEAFF

SEQ ID NO: 29 - protein, 12 aa, synthetic construct
  REGION 1..12: note = Description of Artificial Sequence: Synthetic peptide
CASRKQNYGYTF

SEQ ID NO: 30 - protein, 14 aa, synthetic construct
  REGION 1..14: note = Description of Artificial Sequence: Synthetic peptide
CASSENGGVDEQFF

SEQ ID NO: 31 - protein, 17 aa, synthetic construct
  REGION 1..17: note = Description of Artificial Sequence: Synthetic peptide
CASSSAFTGTEDPGYTF

SEQ ID NO: 32 - protein, 15 aa, synthetic construct
  REGION 1..15: note = Description of Artificial Sequence: Synthetic peptide
CASSEWTSGDNEQFF

SEQ ID NO: 33 - protein, 15 aa, synthetic construct
  REGION 1..15: note = Description of Artificial Sequence: Synthetic peptide
CASSLGTFSTDTQYF

SEQ ID NO: 34 - protein, 15 aa, synthetic construct
  REGION 1..15: note = Description of Artificial Sequence: Synthetic peptide
CASSQGGRGEYEAFF

SEQ ID NO: 35 - protein, 11 aa, synthetic construct
  REGION 1..11: note = Description of Artificial Sequence: Synthetic peptide
CASSPGYEQFF

SEQ ID NO: 36 - protein, 20 aa, synthetic construct
  REGION 1..20: note = Description of Artificial Sequence: Synthetic peptide
CASSHPLGGQGNTWGNEQFF

SEQ ID NO: 37 - protein, 12 aa, synthetic construct
  REGION 1..12: note = Description of Artificial Sequence: Synthetic peptide
CASSFSGTGAFF

SEQ ID NO: 38 - protein, 15 aa, synthetic construct
  REGION 1..15: note = Description of Artificial Sequence: Synthetic peptide
CASSPTGTSGNEQYF

SEQ ID NO: 39 - protein, 14 aa, synthetic construct
  REGION 1..14: note = Description of Artificial Sequence: Synthetic peptide
CASSEGHLNTEAFF

SEQ ID NO: 40 - protein, 12 aa, synthetic construct
  REGION 1..12: note = Description of Artificial Sequence: Synthetic peptide
CASSRVQNEQFF

SEQ ID NO: 41 - protein, 15 aa, synthetic construct
  REGION 1..15: note = Description of Artificial Sequence: Synthetic peptide
CASSFSGTPPQPQHF

SEQ ID NO: 42 - protein, 13 aa, synthetic construct
  REGION 1..13: note = Description of Artificial Sequence: Synthetic peptide
CASSLQGYNEQFF

SEQ ID NO: 43 - protein, 13 aa, synthetic construct
  REGION 1..13: note = Description of Artificial Sequence: Synthetic peptide
CASSIPGKETQYF

SEQ ID NO: 44 - protein, 14 aa, synthetic construct
  REGION 1..14: note = Description of Artificial Sequence: Synthetic peptide
CASSTTLTGIKDTF

SEQ ID NO: 45 - protein, 13 aa, synthetic construct
  REGION 1..13: note = Description of Artificial Sequence: Synthetic peptide
CASSYGLTYEQYF

SEQ ID NO: 46 - protein, 16 aa, synthetic construct
  REGION 1..16: note = Description of Artificial Sequence: Synthetic peptide
CASSSLGDVMNTEAFF

SEQ ID NO: 47 - protein, 13 aa, synthetic construct
  REGION 1..13: note = Description of Artificial Sequence: Synthetic peptide
CASSRGLQPTQYF

SEQ ID NO: 48 - protein, 13 aa, synthetic construct
  REGION 1..13: note = Description of Artificial Sequence: Synthetic peptide
CASSFNPSYEQYF

SEQ ID NO: 49 - protein, 13 aa, synthetic construct
  REGION 1..13: note = Description of Artificial Sequence: Synthetic peptide
CAVKGSDDYKLSF

SEQ ID NO: 50 - protein, 19 aa, synthetic construct
  REGION 1..19: note = Description of Artificial Sequence: Synthetic peptide
CASSPVNLAGVSRADTQYF

SEQ ID NO: 51 - protein, 13 aa, synthetic construct
  REGION 1..13: note = Description of Artificial Sequence: Synthetic peptide
CASSPRGYQPQHF

SEQ ID NO: 52 - protein, 11 aa, synthetic construct
  REGION 1..11: note = Description of Artificial Sequence: Synthetic peptide
CAVTSWGKLQF

SEQ ID NO: 53 - protein, 16 aa, synthetic construct
  REGION 1..16: note = Description of Artificial Sequence: Synthetic peptide
CASSPPEAGLDTEAFF

SEQ ID NO: 54 - protein, 15 aa, synthetic construct
  REGION 1..15: note = Description of Artificial Sequence: Synthetic peptide
CASSLSGGGDYGYTF

SEQ ID NO: 55 - protein, 14 aa, synthetic construct
  REGION 1..14: note = Description of Artificial Sequence: Synthetic peptide
CASGGSGNTGKLIF

SEQ ID NO: 56 - protein, 14 aa, synthetic construct
  REGION 1..14: note = Description of Artificial Sequence: Synthetic peptide
CASSLGQFNYEQYF

SEQ ID NO: 57 - protein, 15 aa, synthetic construct
  REGION 1..15: note = Description of Artificial Sequence: Synthetic peptide
CAMREVLDNTDKLIF

SEQ ID NO: 58 - protein, 14 aa, synthetic construct
  REGION 1..14: note = Description of Artificial Sequence: Synthetic peptide
CSAREQGPLEEQYF

SEQ ID NO: 59 - protein, 14 aa, synthetic construct
  REGION 1..14: note = Description of Artificial Sequence: Synthetic peptide
CASSFGTATYEQYF

SEQ ID NO: 60 - protein, 13 aa, synthetic construct
  REGION 1..13: note = Description of Artificial Sequence: Synthetic peptide
CAMNSGGYQKVTF

SEQ ID NO: 61 - protein, 14 aa, synthetic construct
  REGION 1..14: note = Description of Artificial Sequence: Synthetic peptide
CIVRVAGSARQLTF

SEQ ID NO: 62 - protein, 15 aa, synthetic construct
  REGION 1..15: note = Description of Artificial Sequence: Synthetic peptide
CASSPYRQGSYGYTF

SEQ ID NO: 63 - protein, 14 aa, synthetic construct
  REGION 1..14: note = Description of Artificial Sequence: Synthetic peptide
CAASIPGTASKLTF

SEQ ID NO: 64 - protein, 13 aa, synthetic construct
  REGION 1..13: note = Description of Artificial Sequence: Synthetic peptide
CAASTGNFNKFYF

SEQ ID NO: 65 - protein, 14 aa, synthetic construct
  REGION 1..14: note = Description of Artificial Sequence: Synthetic peptide
CASNRQGTVTEAFF

SEQ ID NO: 66 - protein, 25 aa, synthetic construct
  REGION 1..25: note = Description of Artificial Sequence: Synthetic peptide
ILGDPKKLLTQHFVQENYLEYRQVP